European Patent Specification EP 3 628 326 B1, published February 28, 2024. Title: METHODS AND MATERIALS FOR TREATMENT OF POMPE'S DISEASE. Applicant: Oxyrane UK Limited. The sequence listing filed with the application follows.

SEQUENCE LISTING (12 sequences)

SEQ ID NO: 1 - protein, 898 aa, Homo sapiens
AAQQGASRPGPRDAQAHPGRPRAVPTQCDVPPNSRFDCAPDKAITQEQCEARGCCYIPAKQGLQGAQMGQPWCFFPPSYPSYKLENLSSSEMGYTATLTRTTPTFFPKDILTLRLDVMMETENRLHFTIKDPANRRYEVPLETPHVHSRAPSPLYSVEFSEEPFGVIVRRQLDGRVLLNTTVAPLFFADQFLQLSTSLPSQYITGLAEHLSPLMLSTSWTRITLWNRDLAPTPGANLYGSHPFYLALEDGGSAHGVFLLNSNAMDVVLQPSPALSWRSTGGILDVYIFLGPEPKSVVQQYLDVVGYPFMPPYWGLGFHLCRWGYSSTAITRQVVENMTRAHFPLDVQWNDLDYMDSRRDFTFNKDGFRDFPAMVQELHQGGRRYMMIVDPAISSSGPAGSYRPYDEGLRRGVFITNETGQPLIGKVWPGSTAFPDFTNPTALAWWEDMVAEFHDQVPFDGMWIDMNEPSNFIRGSEDGCPNNELENPPYVPGVVGGTLQAATICASSHQFLSTHYNLHNLYGLTEAIASHRALVKARGTRPFVISRSTFAGHGRYAGHWTGDVWSSWEQLASSVPEILQFNLLGVPLVGADVCGFLGNTSEELCVRWTQLGAFYPFMRNHNSLLSLPQEPYSFSEPAQQAMRKALTLRYALLPHLYTLFHQAHVAGETVARPLFLEFPKDSSTWTVDHQLLWGEALLITPVLQAGKAEVTGYFPLGTWYDLQTVPVEALGSLPPPPAAPREPAIHSEGQWVTLPAPLDTINVHLRAGYIIPLQGPGLTTTESRQQPMALAVALTKGGEARGELFWDDGESLEVLERGAYTQVIFLARNNTIVNELVRVTSEGAGLQLQKVTVLGVATAPQQVLSNGVPVSNFTYSPDTKVLDICVSLLMGEQFLVSWC

SEQ ID NO: 2 - DNA, 5060 bp, Cellulosimicrobium cellulans
atgaaaaagatttggctggcgctggctggtttagttttagcgtttagcgcatcggccggccatcaccatcatcaccacgtggggcccggctcggacgaagtggatgcaccggaacctccgagcgcagattatgcaagcctggttgatgtttttgttggcaccgaaggtgattttggtaatgatatgcctgcagcacaggcaccgaatggtctggcaaaagttaatccgcgtaccacaccgggtcgtaataataccggttatgattatgcccagagcaaaattagcggttttacccataccaatctggatggtgttggtggtagcggtggtggtggtgatctgctggttgttccgaccagcggtagctataccgcacgtccgggtacaggcacctatgcacatccgtttagccatgatgatgaagatgcaggtccgggtttttatagcgttggtctgggtaatgttgcaggcaccgatggtgcaattaccggtgctccgggtacaattgaagcagaagttgcagcagcaacccgtagcggtgttcatcgttatgcatttccggcaggtagcaccccgagcctggttgttgatctggaaaccaataataccagccgtcgtagcagcagcgttcaggttgaaacccgtgcagatggcaccgttgaactgagcggtcaggttaccggctatttttataatgcagcctataccctgtattataccgcacgcaccctgcagcctgcaaccgttcagacctggggtgatgatgatcgtctggttgatgcaaccgcacaggatggtgttgataccggtgcaattctgacctttgatccggcagatgccggtgaaattggtctgcaggttaccctgtctccggttagcgttgaacaggcacgtattgatcagcaggttgaactgggtgatctgagctttgatgcaattcgtgatcgtacccgtgcagaatggaatgcaaccctgggtcgtgttgcaattgatgcaagcaccgcaaccgatccgaccggtgaactgcagcgtctgttttatacccatctgtatcgcatgtttgcaatgccgatgaatgcaaccagcaccagcggcacctatcgtggtgttgatggtgcagttcatgcagcacagggctttacctattatgatagctgggcaacctgggatgattttcgcaaatttagcgtgattgcctatattgatccggcactgtatcgtgatatggttcagagcctggtttacctgtttgcagatgcagaagcaaccggtacaggcggtggtctgggtggttttgttcatagcgttccgaccgttcgttgggaacgtagcagcgttgttgttgcagatgcaattgccaaaggctttgatggttttgatcgtctggatgaagcatatccggcactgcagcgcctggttggtcagtatagcgcagatgaactgcgtcgtggttatgttgcaggtaatccgggtgcaagcgttcagcgtggttatgatcagtatggtctgagcgttattgccgatgaactgggtctgaccgaagaagcagaaaccctgcgcgaacaggcaagctggccgattgaaaaactgaccaaaccgggtgcatggaccgcagcagatggtacacaggttggtctgctgacaccgcgtgcagccgatggtagctggcagagcgcagatcatgccaaatttgaagcagcaggtctgtatcagggcaccctgtggcagtatcattggtatgatgcctatgatatggatgcactggttgaagcaatgggtggtcatgaagcagcccgtctgggtatgcgtcatatgtttggtgaacatgcaccggatgatggtaaagcaatgctgcatagcaatgccaatgaaattgatctgcaggcaccgtacctgtttaattataccggtgaaccgagcctgacccagaaatgggcacgtgcaatttataccaaagaaacctggaatcgctatattgcaaccggtagcagctctgcagttccgtcaggtggtggtgaatttacacctccgctgaaaaccaaagtttatcgtctggaccctcgtggtatgctgccgaccatggataatgatgcaggtacaatgagcaccatgtttgttgcagcagccgttggtctgtttccggttaccgcaggtagcagccagtttcaggttggtagcccgttttttgatagcaccaccattacctatgatgatggtagcgcatttaccgttaccgcagatggtgttagcgaagatgccttttatgttcagagcgcaaccctggatggtgcaacctttggtaatacctgggttgattatgcaaccgttgttggtggtgcagatctggcatttcgtatgggtgaacagccgagcgattggggcaccgataccgcaccggcatttagcatgagcaccgccaccgatgaaccggcagaaggtcctcgcgttagcgcagaaccgaccaccgtgcagaccggtgatggtggtgcactggatgcaaccgttaccctgacactggatggcgcacgtctggcagcaccggcaggtacagatctggttaccagcggtgcagcaagcgttgttggtctgccggatggtgttaccgcagcagttaccgttgcaagcccgaccgcactgaccgttagcctgaccggcaccgcatcagcagatgcacgtttttttgtgcatctgcgtgatgcagcactggccgatggtgttgcagccgcaagcctgcagggtcagggtgttagcgttcgttctccgctgcgtctgagcgttgcaagcgcagaacgtgatgcactggcagcactggttgatgatgccgttctggttcgtcatggtaattatagcagcgttacctttgatcgtttagcaccgctctgacaaaagcacaggaagcactgggcgacgaagcagcaaccagcattgcactgcgttttgcagcagatcgtctgggtgcagcagcagatgcactggatctgaccggtggtggttatcgtaccctggaagcagaacagagcgaagcatggtctggtggtgaactgaaaaatgaagccaatagcagcagcggtaatctgggtggtgttcgtagcggtagctgggttcagtatcgcgatatgacctttgaaaccgcagccggtgatacacctccgcgttttctgaccgttcgttatgataccagctttgcaccgaccgataccccgagcaccgttcgtgttcatgccggtgatgtttctggtccggttgttgcaaccgttgatctgaaaggcaccagcggttggggtaaatataccgaagttaccgcagaactgggtgatgttcaggccctggttgatgcccaggttgttacctttgaactgctggcaccgagcggtcgtagctgggttggtaattttgattggtttcgctttagcgcagaagatccggcagcaccgggtcagcctggtgaaagcccgaccgttaccattgaagccgaagattggaccgcaagcagcggtcgtggtctgaaaaaagaaagcagcacctggaccagcggtccggtgaccaatgttggtggtacagcagatggtgattggattgcctatggtgaagttgatctgggtgaactgccgctgggcgaactgagcgttcattatgtgcataatagcaatcgcagcggtaataatagcgcactgagcgtttatctggatgcatttgatccggctaatccgggtgaaccgtttgttaccgttccgctgccgaccaccggtagcagttggaccgcagatggcacagccaccgttgttctgccggaaaccgtgcagggcacccatgaagtttttgttcgtctgagcaccgaaccgtatgcagatcatccgtatgttgcaaatctggatagcctgacctttgcaccgggtggtccgaccagcgttgtggttgaaagcgaagcctggaccagcaattctggtcgtggcctgaaaaatgaatcttctacctggacctctggtccggttacaaatgtgggtggcaccgctgatggcgattggctggcatatggcgaaattgatctgggcagcgcagcactggatcagctgtctgtgcattatgttcataattctaatcgctctggtcgtaattctgcactgtctgtgtatctggatgcctttgatccggcaaatccgggtgaaccgtttgtgacagtgccgctggcaaataccggtagctcttggaccaccgatggtactgcagttgtggatctgccgtctaccgttcgtggtaaacatcaggtttgggttcgtctgtctaccgaagcatatgccgatcatccgtatgtggccaatctggattctatgcgcttttttaccgatgcatatgatgttgaagttcctccgaccgatacagcagcactggcagccgttgttgatgcagcaggtacaccggaagcagaaattgcacgttatggtcgtattgatgcccgtgtttttacccgtgaactggcagcagcacgtagcgttctggccgatgccggtgcaacacaggcacaggcagatgaacgtgctcgtcgtctgggtctggcaaccgatcagctggttccggcagaacgtcgtcgtctggaaaatctggttgccagcgcagaagcactgaccgacgaaggttattctccggaaagctggcaggcatttcgtaccgcactggctgctgcaaccggcaccctggatgatgcagcagcatctgatgaagcactgcatgatgcacgtctggcgctgcagggtgcagttgatgcactggaagaaccggcagatgttgttctggttgaagttgaagtttctccgcgttgtctggcaggtaaaccgtatgttgccgttcgtgcagttaatgtttctgatgcagccgttgatgttgaactggcaagctctctgggcacccgtagctttgttggtgtggcaccgggtgcgagcgcatatcagagctttgcagcccgtagcgcaaccggtgatctggatgttaccgtgaccgcaaccggtgcagatggtactcagaccgttgaacaggttgtgaccgttccgagctgtagctaataa

SEQ ID NO: 3 - protein, 1665 aa, Cellulosimicrobium cellulans
ALAVVGLAPATAASAAPEPPSADYASLVDVFVGTEGDFGNDMPAAQAPNGLAKVNPRTTPGRNNTGYDYAQSKISGFTHTNLDGVGGSGGGGDLLVVPTSGSYTARPGTGTYAHPFSHDDEDAGPGFYSVGLGNVAGTDGAITGAPGTIEAEVAAATRSGVHRYAFPAGSTPSLVVDLETNNTSRRSSSVQVETRADGTVELSGQVTGYFYNAAYTLYYTARTLQPATVQTWGDDDRLVDATAQDGVDTGAILTFDPADAGEIGLQVTLSPVSVEQARIDQQVELGDLSFDAIRDRTRAEWNATLGRVAIDASTATDPTGELQRLFYTHLYRMFAMPMNATSTSGTYRGVDGAVHAAQGFTYYDSWATWDDFRKFSVIAYIDPALYRDMVQSLVYLFADAEATGTGGGLGGFVHSVPTVRWERSSVVVADAIAKGFDGFDRLDEAYPALQRLVGQYSADELRRGYVAGNPGASVQRGYDQYGLSVIADELGLTEEAETLREQASWPIEKLTKPGAWTAADGTQVGLLTPRAADGSWQSADHAKFEAAGLYQGTLWQYHWYDAYDMDALVEAMGGHEAARLGMRHMFGEHAPDDGKAMLHSNANEIDLQAPYLFNYTGEPSLTQKWARAIYTKETWNRYIATGSSSAVPSGGGEFTPPLKTKVYRLDPRGMLPTMDNDAGTMSTMFVAAAVGLFPVTAGSSQFQVGSPFFDSTTITYDDGSAFTVTADGVSEDAFYVQSATLDGATFGNTWVDYATVVGGADLAFRMGEQPSDWGTDTAPAFSMSTATDEPAEGPRVSAEPTTVQTGDGGALDATVTLTLDGARLAAPAGTDLVTSGAASVVGLPDGVTAAVTVASPTALTVSLTGTASADARFFVHLRDAALADGVAAASLQGQGVSVRSPLRLSVASAERDALAALVDDAVLVRHGNYSSVTFDRFSTALTKAQEALGDEAATSIALRFAADRLGAAADALDLTGGGYRTLEAEQSEAWSGGELKNEANSSSGNLGGVRSGSWVQYRDMTFETAAGDTPPRFLTVRYDTSFAPTDTPSTVRVHAGDVSGPVVATVDLKGTSGWGKYTEVTAELGDVQALVDAQVVTFELLAPSGRSWVGNFDWFRFSAEDPAAPGQPGESPTVTIEAEDWTASSGRGLKKESSTWTSGPVTNVGGTADGDWIAYGEVDLGELPLGELSVHYVHNSNRSGNNSALSVYLDAFDPANPGEPFVTVPLPTTGSSWTADGTATVVLPETVQGTHEVFVRLSTEPYADHPYVANLDSLTFAPGGPTSVVVESEAWTSNSGRGLKNESSTWTSGPVTNVGGTADGDWLAYGEIDLGSAALDQLSVHYVHNSNRSGRNSALSVYLDAFDPANPGEPFVTVPLANTGSSWTTDGTAVVDLPSTVRGKHQVWVRLSTEAYADHPYVANLDSMRFFTDAYDVEVPPTDTAALAAVVDAAGTPEAEIARYGRIDARVFTRELAAARSVLADAGATQAQADERARRLGLATDQLVPAERRRLENLVASAEALTDEGYSPESWQAFRTALAAATGTLDDAAASDEALHDARLALQGAVDALEEPADVVLVEVEVSPRCLAGKPYVAVRAVNVSDAAVDVELASSLGTRSFVGVAPGASAYQSFAARSATGDLDVTVTATGADGTQTVEQVVTVPSCS

SEQ ID NO: 4 - protein, 1650 aa, Cellulosimicrobium cellulans
APEPPSADYASLVDVFVGTEGDFGNDMPAAQAPNGLAKVNPRTTPGRNNTGYDYAQSKISGFTHTNLDGVGGSGGGGDLLVVPTSGSYTARPGTGTYAHPFSHDDEDAGPGFYSVGLGNVAGTDGAITGAPGTIEAEVAAATRSGVHRYAFPAGSTPSLVVDLETNNTSRRSSSVQVETRADGTVELSGQVTGYFYNAAYTLYYTARTLQPATVQTWGDDDRLVDATAQDGVDTGAILTFDPADAGEIGLQVTLSPVSVEQARIDQQVELGDLSFDAIRDRTRAEWNATLGRVAIDASTATDPTGELQRLFYTHLYRMFAMPMNATSTSGTYRGVDGAVHAAQGFTYYDSWATWDDFRKFSVIAYIDPALYRDMVQSLVYLFADAEATGTGGGLGGFVHSVPTVRWERSSVVVADAIAKGFDGFDRLDEAYPALQRLVGQYSADELRRGYVAGNPGASVQRGYDQYGLSVIADELGLTEEAETLREQASWPIEKLTKPGAWTAADGTQVGLLTPRAADGSWQSADHAKFEAAGLYQGTLWQYHWYDAYDMDALVEAMGGHEAARLGMRHMFGEHAPDDGKAMLHSNANEIDLQAPYLFNYTGEPSLTQKWARAIYTKETWNRYIATGSSSAVPSGGGEFTPPLKTKVYRLDPRGMLPTMDNDAGTMSTMFVAAAVGLFPVTAGSSQFQVGSPFFDSTTITYDDGSAFTVTADGVSEDAFYVQSATLDGATFGNTWVDYATVVGGADLAFRMGEQPSDWGTDTAPAFSMSTATDEPAEGPRVSAEPTTVQTGDGGALDATVTLTLDGARLAAPAGTDLVTSGAASVVGLPDGVTAAVTVASPTALTVSLTGTASADARFFVHLRDAALADGVAAASLQGQGVSVRSPLRLSVASAERDALAALVDDAVLVRHGNYSSVTFDRFSTALTKAQEALGDEAATSIALRFAADRLGAAADALDLTGGGYRTLEAEQSEAWSGGELKNEANSSSGNLGGVRSGSWVQYRDMTFETAAGDTPPRFLTVRYDTSFAPTDTPSTVRVHAGDVSGPVVATVDLKGTSGWGKYTEVTAELGDVQALVDAQVVTFELLAPSGRSWVGNFDWFRFSAEDPAAPGQPGESPTVTIEAEDWTASSGRGLKKESSTWTSGPVTNVGGTADGDWIAYGEVDLGELPLGELSVHYVHNSNRSGNNSALSVYLDAFDPANPGEPFVTVPLPTTGSSWTADGTATVVLPETVQGTHEVFVRLSTEPYADHPYVANLDSLTFAPGGPTSVVVESEAWTSNSGRGLKNESSTWTSGPVTNVGGTADGDWLAYGEIDLGSAALDQLSVHYVHNSNRSGRNSALSVYLDAFDPANPGEPFVTVPLANTGSSWTTDGTAVVDLPSTVRGKHQVWVRLSTEAYADHPYVANLDSMRFFTDAYDVEVPPTDTAALAAVVDAAGTPEAEIARYGRIDARVFTRELAAARSVLADAGATQAQADERARRLGLATDQLVPAERRRLENLVASAEALTDEGYSPESWQAFRTALAAATGTLDDAAASDEALHDARLALQGAVDALEEPADVVLVEVEVSPRCLAGKPYVAVRAVNVSDAAVDVELASSLGTRSFVGVAPGASAYQSFAARSATGDLDVTVTATGADGTQTVEQVVTVPSCS

SEQ ID NO: 5 - protein, 1079 aa, Yarrowia lipolytica
MYSHFNNEPVAKRVNNLFTDRLRQFTSDGEYRSLNLPAFYERERLDGKNHVAIETYAVSDLRRPLFKDALKEADGHWKPAKKGSEYGPSWATHWFKIQVCVPPEWKKNYYKKGDLVVFNWNLNCEGLVFSESGEALIGLSGEERREWPIPDNWFDGKCHTFYIEASCNGMFGNATGSSIQPPSDNRYFRLDSADLVVINSEARHLFVDFWIIGDAAREFPGDSWQRGKALDVANKIMDAFDPENPDESIAEGRKLAKEYLGDTTKAYKQQLPFADGLVYALGNCHIDTAWLWPFAETRRKAGRSWASQLELIDKYPEYVFVASQAQQFKWLKEDYPDLFAKIQKQAKKGRFLPVGGAWTECDTNLPSGESLLRQFLLGQRFFLEHFGSLSDTFWLPDTFGYSAQVPQLCRLAGMDRFLTQKLSWNNINSFPNSTFNWVALDGSQVLCHMPPNNTYTSMANFGDVSRTQKQNKNLDTTRNSLMLYGHGDGGGGPTAEMLEKLRRCRGVSNTVGELPPVIQGQSVTDFYNELLDQTNNGKDLVTWVGELYFEFHRGTYTSQAQTKKGNRVSENLLHDVELLATLASIRDSSYKYPFAQLESLWEDVCLCQFHDVLPGSCIEMVYKDVKKIHGRVIDTASHLIDKAASALGLSGHPSKDSFDCTPVALNTMPWSRTEVVAVPQPHWDATVELAEGVEIQEDSGNALVMMSESGPVVTTQSVDLFKSEDAYILENSQVKVTICKDDGTLTSIYDKENDRRVLSGTGNRLVLFDDQPLSWQAWDTEVFSLGKKQYIGAENVTRHSIVSSGPLRSTVAFTYEFNKSVVTTEISLDANSPLVTFNTRADWHETCKFLKVEFPVDVHSESASYESQFGVVKRPTHYNTSWDVAKFEVCCHKFADLSELDYGVSILNDCKYGFATHGNLMRLSLLRAPKAPDAHADMGHHEFKYGVLAHKGPLGATTVRAAYNFNNPLRVKYVGLSEVSTKQAFSLKGPANLVLSQVKRAEVDRSKKSTNVILRVYEALGGRTRGKLVIDLPNVVSVTKTCALEYSKEKQVVAKSEGVTSVDISLRAFEVATYKVELA

SEQ ID NO: 6 - protein, 513 aa, Aspergillus satoi
MHLPSLSLSLTALAIASPSAAYPHFGSSQPVLHSSSDTTQSRADAIKAAFSHAWDGYLQYAFPHDELHPVSNGYGDSRNGWGASAVDALSTAVIMRNATIVNQILDHVGKIDYSKTNTTVSLFETTIRYLGGMLSGYDLLKGPVSDLVQNSSKIDVLLTQSKNLADVLKFAFDTPSGVPYNNLNITSGGNDGAKTNGLAVTGTLALEWTRLSDLTGDTTYADLSQKAESYLLNPQPKSAEPFPGLVGSNINISNGQFTDAQVSWNGGDDSYYEYLIKMYVYDPKRFGLYKDRWVAAAQSTMQHLASHPSSRPDLTFLASYNNGTLGLSSQHLTCFDGGSFLLGGTVLNRTDFINFGLDLVSGCHDTYNSTLTGIGPESFSWDTSDIPSSQQSLYEKAGFYITSGAYILRPEVIESFYYAWRVTGQETYRDWIWSAFSAVNDYCRTSSGFSGLTDVNAANGGSRYDNQESFLFAEVMKYSYMAFAEDAAWQVQPGSGNQFVFNTEAHPVRVSST

SEQ ID NO: 7 - protein, 1810 aa, Cellulosimicrobium cellulans
MTRPLPPGRAVARSGSGRARPLGLVLAAALAVPLGVPLAAPAGALAAAPAAAAEPGDFSSSFESGDPAALPTTVAERDGAPWQANVGSFTAGLPGSVLGQLKGVTASAQNLPNEGAANLADGSSGTKWLAFASTGWVRYEFAEPVSFVAYTMTSGDDAAGRDPKTWTVEGSNDGSTWAALDRRTDEDFPNRQQTRTFELEAPTAAYTYLRLNVTANSGDSIVQLAGWDLSADLSAGPSAAPMTTKVGTGPRVSFTNKAGVGFSGLHSLRYDGSHLADGETYATNVLYDDVDVVVGEDTRLSYTIFPELLDDLQYPSTYAAVDVLFTDGTYLSDLGARDAHETVATAQAQGEGKILYADQWNSVRVDLGDVAEGKTVDQVLLGYDNPGGHAGTKFAGWLDDVEITAEPATIDGSSLANYVDTRRGTLASGSFSRGNNIPATATPNGFNFWTPYTNASSQSWLYEYHKANNANNKPVLQGFGISHEPSPWMGDRNQLTFLPSTASGTPDATLSTRGLEFDHADETARPDYYGVTFTNGSAIEATPTDHGAVLRFSYPGAKGHVLVDKVDGSSKLTYDQATGTISGWVENGSGLSVGRTRMFVAGTFDRSPTAVGTAAGNRADARFATFETSSDKTVELRVATSFISLDQARKNLDLEVTGKTFTEVKAAAAQAWNDRLGVIEVEGASEDQLVTLYSNLYRLNLYPNSQFENTGTAQEPVYRYASPVSATTGSATDTQTNAKIVDGKIYVNNGFWDTYRTAWPAYSLLYPELAAELVDGFVQQYRDGGWIARWSSPGYADLMTGTSSDVAFADAYLKGSLPTGTALEAYDAALRNATVAPPSNAVGRKGLQTSPFLGFTPESTHESVSWGLEGLVNDFGIGNMAAALAEDPATPEERRETLREESAYFLERATHYVELFDPEVDFFVPRHEDGTWAVDPETYDPEAWGGGYTETNGWNFAFHAPQDGQGLANLYGGKQGLEDKLDEFFSTPEKGAGNGGIHEQREARDVRMGQWGMSNQVSHHIPWLYDAAGAPSKAQEKVREVTRRLFVGSEIGQGYPGDEDNGEMSSWWIFASLGFYPLQVGSDQYAVGSPLFDKATVHLPDGDLVVNAENNSVDNVYVQSLAVDGEARTSTSLSQADLSGGTTLDFVMGPEPSDWGTGEDDAPPSLTEGDEPPTPVQDATTAGLGTTTVADGDATTSAAALTDNTSGTRTTFATTTPSITWAGNGIRPTVGSYTLTSGASGTASPSAWTLEGSDDGETWTTLDERSGEQFRWALQTRPFTVAEPTAFARYRVTVTATSGSGALSLAEVELLADPKESGAEELTLSAAPDRDGVTGREVSGSFATLTGVEGDVAALDVQVAFGDGSEPVAGTLRAGAFGGYAVDAAHTWTAPGVYPVTVTVSGEGIETVSASSYVSVSLLREGSLLAAYDNVCIGDAGTTVGSCDGQGVFFDRAQLAAKGFVQGERATVPGTDLAFDVPAVPAGQPDNATGDGQTIELDVPADAEQLSVIGTGTEKNQQATGTLTFDDGSTQPIDLSFGDWSGAARNPVFGNIPVAVTDSRLRGGSPQTGTPAAFFATAPITLPEGKRPVSLTLPDQPGELSRDGRIHVVAVAHDGTFAEHPALEVTAAEGVTLAVGQTSDVALAQVAGGREGADLRAAVTWGDGSDVAAGAVTDGSVSGSHAYTAAGTYTAYVVVDDGWTSQVVEVPVTVTEAEPALAVDVTVSTRCLAGKAYVAVRAENGEDVPLAIRLVTPFGTKEVAAVAPGANAYSFATRVTAVEAGTVTVEATRGTGDEEVTASIQADYAAVTCG

SEQ ID NO: 8 - protein, 282 aa, Aspergillus oryzae
GLTTQKSAPWGLGSISHKGQQSTDYIYDTSAGEGTYAYVVDSGVNVDHEEFEGRASKAYNAAGGQHVDSIGHGTHVSGTIAGKTYGIAKKASILSVKVFQGESSSTSVILDGFNWAANDIVSKKRTSKAAINMSLGGGYSKAFNDAVENAFEQGVLSVVAAGNENSDAGQTSPASAPDAITVAAIQKSNNRASFSNFGKVVDVFAPGQDILSAWIGSSSATNTISGTSMATPHIVGLSLYLAALENLDGPAAVTKRIKELATKDVVKDVKGSPNLLAYNGNA

SEQ ID NO: 9 - protein, 403 aa, Aspergillus oryzae
MQSIKRTLLLLGAILPAVLGAPVQETRRAAEKLPGKYIVTFKPGIDEAKIQEHTTWATNIHQRSLERRGATGGDLPVGIERNYKINKFAAYAGSFDDATIEEIRKNEDVAYVEEDQIYYLDGLTTQKSAPWGLGSISHKGQQSTDYIYDTSAGEGTYAYVVDSGVNVDHEEFEGRASKAYNAAGGQHVDSIGHGTHVSGTIAGKTYGIAKKASILSVKVFQGESSSTSVILDGFNWAANDIVSKKRTSKAAINMSLGGGYSKAFNDAVENAFEQGVLSVVAAGNENSDAGQTSPASAPDAITVAAIQKSNNRASFSNFGKVVDVFAPGQDILSAWIGSSSATNTISGTSMATPHIVGLSLYLAALENLDGPAAVTKRIKELATKDVVKDVKGSPNLLAYNGNA

SEQ ID NO: 10 - DNA, 1272 bp, Artificial sequence
  codon optimized sequence encoding alkaline protease
ggatccatgcagtccattaagcgaactctgctgctgctgggagccattctgcccgccgtgctgggagcccccgttcaggagacccgacgagccgccgagaagctccccggcaagtacattgtcaccttcaagcctggtatcgacgaggctaagattcaggagcacaccacttgggccaccaacatccatcagcgatccctcgagcgacgaggagccaccggcggtgacctgcctgtgggaatcgagcgaaactacaagattaacaagttcgccgcttacgctggatcttttgacgatgccaccatcgaggagattcgaaagaacgaggacgtcgcttacgtggaggaagaccagatctactacctcgatggtctgaccactcagaagtccgctccttggggcctgggctccatctctcacaagggacagcagtcgactgactacatctacgatacctccgctggcgagggtacttacgcctacgtcgtggactccggtgttaacgtcgatcacgaggagtttgagggacgagcctctaaggcttacaacgccgctggaggccagcatgtggactctatcggacacggcacccatgtttcgggtactattgccggaaagacctacggcatcgccaagaaggcttctattctctcggtgaaggttttccagggagagtcctcttcgacctctgtcatcctggacggctttaactgggccgctaacgatattgtgtctaagaagcgaacctcgaaggccgctatcaacatgtccctcggtggaggctactctaaggccttcaacgacgctgttgagaacgcctttgagcagggtgtcctgtctgttgtggctgctggtaacgagaactctgacgctggacagacctcccctgcttctgctcctgatgccatcactgtggccgctattcagaagtccaacaaccgagcttcgttctccaactttggcaaggtggttgacgttttcgcccccggacaggatatcctctctgcttggattggctcctcttcggccaccaacactatctcgggcacctccatggccactccccacattgtcggtctgtccctctacctggctgctctggagaacctggacggacctgccgctgttaccaagcgaatcaaggagctggctactaaggacgtcgtgaaggatgtcaagggttctcctaacctgctcgcctacaacggcaacgcttctggcggcggaggacatcaccaccatcaccatcaccaccatcattgataacctagg

SEQ ID NO: 11 - protein, 20 aa, Artificial sequence
  peptide from Jack bean mannosidase
NKIPRAGWQIDPFGHSAVQG

SEQ ID NO: 12 - protein, 7 aa, Artificial sequence
  alkaline protease substrate
IQNCPLG